European Patent Application EP 4 442 805 A1, published October 9, 2024. Title: 엔테로코커스 패시움 LCM001 균주를 포함하는 생리전증후군 완화 또는 치료용 약학적 조성물. Applicant: 주식회사 엠바이옴쎄라퓨틱스. The sequence listing filed with the application follows.

SEQUENCE LISTING (1 sequence)

SEQ ID NO: 1 - DNA, 1457 bp, Enterococcus faecium
  source 1..1457: mol_type = genomic DNA
gttggatcttggatcaggacgaacgctggcggcgtgcctaatacatgcaagtcgtacgcttctttttccaccggagcttgctccaccggaaaaagaagagtggcgaacgggtgagtaacacgtgggtaacctgcccatcagaaggggataacacttggaaacaggtgctaataccgtataacaatcgaaaccgcatggttttgatttgaaaggcgctttcgggtgtcgctgatggatggacccgcggtgcattagctagttggtgaggtaacggctcaccaaggccacgatgcatagccgacctgagagggtgatcggccacattgggactgagacacggcccaaactcctacgggaggcagcagtagggaatcttcggcaatggacgaaagtctgaccgagcaacgccgcgtgagtgaagaaggttttcggatcgtaaaactctgttgttagagaagaacaaggatgagagtaactgttcatcccttgacggtatctaaccagaaagccacggctaactacgtgccagcagccgcggtaatacgtaggtggcaagcgttgtccggatttattgggcgtaaagcgagcgcaggcggtttcttaagtctgatgtgaaagcccccggctcaaccggggagggtcattggaaactgggagacttgagtgcagaagaggagagtggaattccatgtgtagcggtgaaatgcgtagatatatggaggaacaccagtggcgaaggcggctctctggtctgtaactgacgctgaggctcgaaagcgtggggagcaaacaggattagataccctggtagtccacgccgtaaacgatgagtgctaagtgttggagggtttccgcccttcagtgctgcagctaacgcattaagcactccgcctggggagtacgaccgcaaggttgaaactcaaaggaattgacgggggcccgcacaagcggaggagcctgtggtttaattcgaaccaacgcgaacaaccttaccaggtcttgacatcctttgaccactccagagatagaccttccccttcgggggcaaagtgacaggtggtgcatggttgtcgtcagctcgtgtcgtgagatgttgggttaagtcccgcaacgagcgcaacccttattgttagttgccatcattcagttgggcactctagcaagactgccggtgacaaaccggaggaaggtggggatgacgtcaaatcatcatgccccttatgacctgggctacacacgtgctacaatgggaagtacaacgagttgcgaagtcgcgaggctaagctaatctcttaaagcttctctcagttcggattgcaggctgcaactcgcctgcatgaagccggaatcgctagtaatcgcggatcagcacgccgcggtgaatacgttcccgggccttgtacacaccgcccgtcacaccacgagagtttgtaacaccagatgtcggtgaggtaacc